European Patent Specification EP 3 511 004 B1, published July 3, 2024. Title: Combined Preparations for the Treatment of Cancer. Applicant: Immutep S.A.S. Application Divisional of EP14830806.7. The sequence listing filed with the application follows.

SEQUENCE LISTING (2 sequences)

SEQ ID NO: 1 - protein, 502 aa, Homo sapiens
LQPGAEVPVVWAQEGAPAQLPCSPTIPLQDLSLLRRAGVTWQHQPDSGPPAAAPGHPLAPGPHPAAPSSWGPRPRRYTVLSVGPGGLRSGRLPLQPRVQLDERGRQRGDFSLWLRPARRADAGEYRAAVHLRDRALSCRLRLRLGQASMTASPPGSLRASDWVILNCSFSRPDRPASVHWFRNRGQGRVPVRESPHHHLAESFLFLPQVSPMDSGPWGCILTYRDGFNVSIMYNLTVLGLEPPTPLTVYAGAGSRVGLPCRLPAGVGTRSFLTAKWTPPGGGPDLLVTGDNGDFTLRLEDVSQAQAGTYTCHIHLQEQQLNATVTLAIITVTPKSFGSPGSLGKLLCEVTPVSGQERFVWSSLDTPSQRSFSGPWLEAQEAQLLSQPWQCQLYQGERLLGAAVYFTELSSPGAQRSGRAPGALPAGHLLLFLTLGVLSLLLLVTGAFGFHLWRRQWRPRRFSALEQGIHPQAQSKIEELEQEPEPEPEPEPEPEPEPEPEQL

SEQ ID NO: 2 - protein, 30 aa, Homo sapiens
GPPAAAPGHPLAPGPHPAAPSSWGPRPRRY